European Patent Application EP 4 524 260 A2, published March 19, 2025. Title: Combined Solution Phase and Solid Phase DNA Amplification. Applicant: DNAe Diagnostics Limited. Application EP 23185680.8, filed July 14, 2023. The sequence listing filed with the application follows.

SEQUENCE LISTING (20 sequences)

SEQ ID NO: 1 - DNA, 18 bp, synthetic construct
  source 1..18: mol_type = other DNA
agcccagaacctgaatcg

SEQ ID NO: 2 - DNA, 20 bp, synthetic construct
  source 1..20: mol_type = other DNA
ccctactcatcgaactcacg

SEQ ID NO: 3 - DNA, 20 bp, synthetic construct
  source 1..20: mol_type = other DNA
  misc_feature <1: note = The C at position 1 is attached to Spacer 18, which is an 18-atom hexa-ethyleneglycol spacer (iSp18), which is attached to an amino modifier with six carbons (5AmMC6)
ccctactcatcgaactcacg

SEQ ID NO: 4 - DNA, 20 bp, synthetic construct
  source 1..20: mol_type = other DNA
  misc_feature <1: note = The T at position 1 is attached to Spacer 18, which is an 18-atom hexa-ethyleneglycol spacer (iSp18), which is attached to an amino modifier with six carbons (5AmMC6)
tgtgtgttagtggaagcgtc

SEQ ID NO: 5 - DNA, 20 bp, synthetic construct
  source 1..20: mol_type = other DNA
  misc_feature <1: note = The G at position 1 is attached to Spacer 18, which is an 18-atom hexa-ethyleneglycol spacer (iSp18), which is attached to an amino modifier with six carbons (5AmMC6)
gggaggttcagttactaacg

SEQ ID NO: 6 - DNA, 20 bp, synthetic construct
  source 1..20: mol_type = other DNA
  misc_feature <1: note = The G at position 1 is attached to Spacer 18, which is an 18-atom hexa-ethyleneglycol spacer (iSp18), which is attached to an amino modifier with six carbons (5AmMC6)
gatcgtaaaactctgttgtt

SEQ ID NO: 7 - DNA, 99 bp, synthetic construct
  source 1..99: mol_type = other DNA
  misc_feature <1: note = The T at position 1 is attached to an amino modifier with six carbons (5AmMC6)
tttttttttttttttcgcgcttcaattccttgttcaacgattgctcgagaatcatactgataggctgttgctaaagcattttgcagctcttctcggttt

SEQ ID NO: 8 - DNA, 20 bp, synthetic construct
  source 1..20: mol_type = other DNA
  misc_feature <1: note = The T at position 1 is attached to a fluorescent dye (5 Cy3)
tgtgtgttagtggaagcgtc

SEQ ID NO: 9 - DNA, 24 bp, synthetic construct
  source 1..24: mol_type = other DNA
ttcagtgagttctcctgttgattg

SEQ ID NO: 10 - DNA, 23 bp, synthetic construct
  source 1..23: mol_type = other DNA
aacgttggtataggagaatgaag

SEQ ID NO: 11 - DNA, 62 bp, synthetic construct
  source 1..62: mol_type = other DNA
  misc_feature 20^21: note = In between the C at position 20 and the A at position 21 is Spacer 18, which is an 18-atom hexa-ethyleneglycol spacer (iSp18)
ttttttttttccccccccccaatactattaatatcacctcagtttcagctgggactaatgaa

SEQ ID NO: 12 - DNA, 63 bp, synthetic construct
  source 1..63: mol_type = other DNA
  misc_feature 20^21: note = In between the C at position 20 and the G at position 21 is Spacer 18, which is an 18-atom hexa-ethyleneglycol spacer (iSp18)
ttttttttttccccccccccgggactaatgaattgtttttacctactttatcccatgctcacg

SEQ ID NO: 13 - DNA, 58 bp, synthetic construct
  source 1..58: mol_type = other DNA
  misc_feature 20^21: note = In between the C at position 20 and the C at position 21 is Spacer 18, which is an 18-atom hexa-ethyleneglycol spacer (iSp18)
ttttttttttccccccccccccatacacagacataagatataacggcttcccagaacc

SEQ ID NO: 14 - DNA, 61 bp, synthetic construct
  source 1..61: mol_type = other DNA
  misc_feature 20^21: note = In between the C at position 20 and the G at position 21 is Spacer 18, which is an 18-atom hexa-ethyleneglycol spacer (iSp18)
ttttttttttccccccccccgagcatattatcctttaataccattcgtttaatcccgtcca

SEQ ID NO: 15 - DNA, 62 bp, synthetic construct
  source 1..62: mol_type = other DNA
  misc_feature 20^21: note = In between the C at position 20 and the A at position 21 is Spacer 18, which is an 18-atom hexa-ethyleneglycol spacer (iSp18)
ttttttttttccccccccccagtctaagtagctcagcaaatgcatcacaaacagataacggc

SEQ ID NO: 16 - DNA, 61 bp, synthetic construct
  source 1..61: mol_type = other DNA
  misc_feature 20^21: note = In between the C at position 20 and the G at position 21 is Spacer 18, which is an 18-atom hexa-ethyleneglycol spacer (iSp18)
ttttttttttccccccccccgataacggcgtaaatagaagtggttctgaagatccaacagt

SEQ ID NO: 17 - DNA, 63 bp, synthetic construct
  source 1..63: mol_type = other DNA
  misc_feature 20^21: note = In between the C at position 20 and the T at position 21 is Spacer 18, which is an 18-atom hexa-ethyleneglycol spacer (iSp18)
ttttttttttccccccccccttagactattattggttgatacacctgaaacaaagcatcctaa

SEQ ID NO: 18 - DNA, 62 bp, synthetic construct
  source 1..62: mol_type = other DNA
  misc_feature 20^21: note = In between the C at position 20 and the A at position 21 is Spacer 18, which is an 18-atom hexa-ethyleneglycol spacer (iSp18)
ttttttttttccccccccccaggtgtagagaaatatggtcctgaagcaagtgcatttacgaa

SEQ ID NO: 19 - DNA, 99 bp, synthetic construct
  source 1..99: mol_type = other DNA
ttttttttttccccccccccttcaattccttgttcaacgattgctcgagaatcatactgataggctgttgctaaagcattttgcagctcttctcggttt

SEQ ID NO: 20 - DNA, 23 bp, synthetic construct
  source 1..23: mol_type = other DNA
  misc_feature <1: note = The C at position 1 is attached to a fluorescent dye (5 Cy3).
ctgcgcgtttacctactttgact